European Patent Specification EP 3 436 484 B1, published October 1, 2025. Title: Recombinant Intravenous Immunoglobulin (rIVIG) Compositions  and Methods for Their Production and Use. Applicant: AB Biosciences, Inc. Hsu, Yen-Ming. Application 62/315,483. The sequence listing filed with the application follows.

SEQUENCE LISTING (10 sequences)

SEQ ID NO: 1 - protein, 375 aa, Artificial Sequence
  Synthesized
DKTHTCPPCPAPELLGGPSVFLFPPKPKDTLMISRTPEVTCVVVDVSHEDPEVKFNWYVDGVEVHNAKTKPREEQYNSTYRVVSVLTVLHQDWLNGKEYKCKVSNKALPAPIEKTISKAKGQPREPQVYTLPPSRDELTKNQVSLTCLVKGFYPSDIAVEWESNGQPENNYKTTPPVLDSDGSFFLYSKLTVDKSRWQQGNVFSCSVMHEALHNHYTQKSLSLSPGGILGDQNPQIAAHVISEASSKTTSVLQWAEKGYYTMSNNLVTLENGKQLTVKRQGLYYIYAQVTFCSNREASSQAPFIASLCLKSPGRFERILLRAANTHSSAKPCGQQSIHLGGVFELQPGASVFVNVTDPSQVSHGTGFTSFGLLKL

SEQ ID NO: 2 - protein, 519 aa, Artificial Sequence
  Synthesized
APELLGGPSVFLFPPKPKDTLMISRTPEVTCVVVDVSHEDPEVKFNWYVDGVEVHNAKTKPREEQYNSTYRVVSVLTVLHQDWLNGKEYKCKVSNKALPAPIEKTISKAKGQPREPQVYTLPPSRDELTKNQVSLTCLVKGFYPSDIAVEWESNGQPENNYKTTPPVLDSDGSFFLYSKLTVDKSRWQQGNVFSCSVMHEALHNHYTQKSLSLSPGGGGGSGGGGSGGGGSGGGGSGGGGSAPELLGGPSVFLFPPKPKDTLMISRTPEVTCVVVDVSHEDPEVKFNWYVDGVEVHNAKTKPREEQYNSTYRVVSVLTVLHQDWLNGKEYKCKVSNKALPAPIEKTISKAKGQPREPQVYTLPPSRDELTKNQVSLTCLVKGFYPSDIAVEWESNGQPENNYKTTPPVLDSDGSFFLYSKLTVDKSRWQQGNVFSCSVMHEALHNHYTQKSLSLSPGGGGGSGPPGISGPPGDPGLPGKDGDHGKPGIQGQPGPPGICDPSLCFSVIARRDPFRKGPNY

SEQ ID NO: 3 - protein, 509 aa, Artificial Sequence
  Synthesized
APELLGGPSVFLFPPKPKDTLMISRTPEVTCVVVDVSHEDPEVKFNWYVDGVEVHNAKTKPREEQYNSTYRVVSVLTVLHQDWLNGKEYKCKVSNKALPAPIEKTISKAKGQPREPQVYTLPPSRDELTKNQVSLTCLVKGFYPSDIAVEWESNGQPENNYKTTPPVLDSDGSFFLYSKLTVDKSRWQQGNVFSCSVMHEALHNHYTQKSLSLSPGGGGGSGGGGSGGGGSAPELLGGPSVFLFPPKPKDTLMISRTPEVTCVVVDVSHEDPEVKFNWYVDGVEVHNAKTKPREEQYNSTYRVVSVLTVLHQDWLNGKEYKCKVSNKALPAPIEKTISKAKGQPREPQVYTLPPSRDELTKNQVSLTCLVKGFYPSDIAVEWESNGQPENNYKTTPPVLDSDGSFFLYSKLTVDKSRWQQGNVFSCSVMHEALHNHYTQKSLSLSPGGGGGSGPPGISGPPGDPGLPGKDGDHGKPGIQGQPGPPGICDPSLCFSVIARRDPFRKGPNY

SEQ ID NO: 4 - protein, 768 aa, Artificial Sequence
  Synthesized
VEIKRTVAAPSVFIFPPSDEQLKSGTASVVCLLNNFYPREAKVQWKVDNALQSGNSQESVTEQDSKDSTYSLSSTLTLSKADYEKHKVYACEVTHQGLSSPVTKSFNRGECGGGGSGGGGSASTKGPSVFPLAPSSKSTSGGTAALGCLVKDYFPEPVTVSWNSGALTSGVHTFPAVLQSSGLYSLSSVVTVPSSSLGTQTYICNVNHKPSNTKVDKRVEPKSCDKTHTCPPCPAPELLGGPSVFLFPPKPKDTLMISRTPEVTCVVVDVSHEDPEVKFNWYVDGVEVHNAKTKPREEQYNSTYRVVSVLTVLHQDWLNGKEYKCKVSNKALPAPIEKTISKAKGQPREPQVYTLPPSRDELTKNQVSLTCLVKGFYPSDIAVEWESNGQPENNYKTTPPVLDSDGSFFLYSKLTVDKSRWQQGNVFSCSVMHEALHNHYTQKSLSLSPGGGGGSGGGGSGGGGSGGGGSGGGGSEPKSCDKTHTCPPCPAPELLGGPSVFLFPPKPKDTLMISRTPEVTCVVVDVSHEDPEVKFNWYVDGVEVHNAKTKPREEQYNSTYRVVSVLTVLHQDWLNGKEYKCKVSNKALPAPIEKTISKAKGQPREPQVYTLPPSRDELTKNQVSLTCLVKGFYPSDIAVEWESNGQPENNYKTTPPVLDSDGSFFLYSKLTVDKSRWQQGNVFSCSVMHEALHNHYTQKSLSLSPGGGGGSGPPGISGPPGDPGLPGKDGDHGKPGIQGQPGPPGICDPSLCFSVIARRDPFRKGPNY

SEQ ID NO: 5 - protein, 549 aa, Artificial Sequence
  Synthesized
EPKSCDKTHTCPPCPAPELLGGPSVFLFPPKPKDTLMISRTPEVTCVVVDVSHEDPEVKFNWYVDGVEVHNAKTKPREEQYNSTYRVVSVLTVLHQDWLNGKEYKCKVSNKALPAPIEKTISKAKGQPREPQVYTLPPSRDELTKNQVSLTCLVKGFYPSDIAVEWESNGQPENNYKTTPPVLDSDGSFFLYSKLTVDKSRWQQGNVFSCSVMHEALHNHYTQKSLSLSPGGGGGSGGGGSGGGGSGGGGSGGGGSEPKSCDKTHTCPPCPAPELLGGPSVFLFPPKPKDTLMISRTPEVTCVVVDVSHEDPEVKFNWYVDGVEVHNAKTKPREEQYNSTYRVVSVLTVLHQDWLNGKEYKCKVSNKALPAPIEKTISKAKGQPREPQVYTLPPSRDELTKNQVSLTCLVKGFYPSDIAVEWESNGQPENNYKTTPPVLDSDGSFFLYSKLTVDKSRWQQGNVFSCSVMHEALHNHYTQKSLSLSPGGGGGSGPPGISGPPGDPGLPGKDGDHGKPGIQGQPGPPGICDPSLCFSVIARRDPFRKGPNY

SEQ ID NO: 6 - protein, 796 aa, Artificial Sequence
  Synthesized
ETVTCEDAQKTCPAVIACSSPGINGFPGKDGRDGTKGEKGEPGQGLRGLQGPPGKLGPPGNPGPSGSPGPKGQKGDPGKGGGGSGGGGSGGGGSRTVAAPSVFIFPPSDEQLKSGTASVVCLLNNFYPREAKVQWKVDNALQSGNSQESVTEQDSKDSTYSLSSTLTLSKADYEKHKVYACEVTHQGLSSPVTKSFNRGECGGGGSGGGGSASTKGPSVFPLAPSSKSTSGGTAALGCLVKDYFPEPVTVSWNSGALTSGVHTFPAVLQSSGLYSLSSVVTVPSSSLGTQTYICNVNHKPSNTKVDKRVEPKSCDKTHTCPPCPAPELLGGPSVFLFPPKPKDTLMISRTPEVTCVVVDVSHEDPEVKFNWYVDGVEVHNAKTKPREEQYNSTYRVVSVLTVLHQDWLNGKEYKCKVSNKALPAPIEKTISKAKGQPREPQVYTLPPSRDELTKNQVSLTCLVKGFYPSDIAVEWESNGQPENNYKTTPPVLDSDGSFFLYSKLTVDKSRWQQGNVFSCSVMHEALHNHYTQKSLSLSPGGGGGSGGGGSGGGGSGGGGSGGGGSEPKSCDKTHTCPPCPAPELLGGPSVFLFPPKPKDTLMISRTPEVTCVVVDVSHEDPEVKFNWYVDGVEVHNAKTKPREEQYNSTYRVVSVLTVLHQDWLNGKEYKCKVSNKALPAPIEKTISKAKGQPREPQVYTLPPSRDELTKNQVSLTCLVKGFYPSDIAVEWESNGQPENNYKTTPPVLDSDGSFFLYSKLTVDKSRWQQGNVFSCSVMHEALHNHYTQKSLSLSPG

SEQ ID NO: 7 - protein, 802 aa, Artificial Sequence
  Synthesized
DKEALSEAQRTCPVVTCALPGRDGRDGLKGEKGEPGQGLRGLQGPPGKVGPPGNTGAPGAPGLKGHKGDRGDGGGGSGGGGSGGGGSRNDAQPAVYLFQPSPDQLHTGSASVVCLLNSFYPKDINVKWKVDGVIQDTGIQESVTEQDKDSTYSLSSTLTMSSTEYLSHELYSCEITHKSLPSTLIKSFQRSECQRVDGGGGSGGGGSASTTAPSVFPLAPSCGSTSGSTVALACLVSGYFPEPVTVSWNSGSLTSGVHTFPSVLQSSGLYSLSSMVTVPSSRWPSETFTCNVAHPASKTKVDKPVPKRENGRVPRPPDCPKCPAPEMLGGPSVFIFPPKPKDTLLIARTPEVTCVVVDLDPEDPEVQISWFVDGKQMQTAKTQPREEQFNGTYRVVSVLPIGHQDWLKGKQFTCKVNNKALPSPIERTISKARGQAHQPSVYVLPPSREELSKNTVSLTCLIKDFFPPDIDVEWQSNGQQEPESKYRTTPPQLDEDGSYFLYSKLSVDKSRWQRGDTFICAVMHEALHNHYTQKSLSHSPGGGGGSGGGGSGGGGSGGGGSGGGGSPKRENGRVPRPPDCPKCPAPEMLGGPSVFIFPPKPKDTLLIARTPEVTCVVVDLDPEDPEVQISWFVDGKQMQTAKTQPREEQFNGTYRVVSVLPIGHQDWLKGKQFTCKVNNKALPSPIERTISKARGQAHQPSVYVLPPSREELSKNTVSLTCLIKDFFPPDIDVEWQSNGQQEPESKYRTTPPQLDEDGSYFLYSKLSVDKSRWQRGDTFICAVMHEALHNHYTQKSLSHSPG

SEQ ID NO: 8 - protein, 779 aa, Artificial Sequence
  Synthesized
RNDAQPAVYLFQPSPDQLHTGSASVVCLLNSFYPKDINVKWKVDGVIQDTGIQESVTEQDKDSTYSLSSTLTMSSTEYLSHELYSCEITHKSLPSTLIKSFQRSECQRVDGGGGSGGGGSASTTAPSVFPLAPSCGSTSGSTVALACLVSGYFPEPVTVSWNSGSLTSGVHTFPSVLQSSGLYSLSSMVTVPSSRWPSETFTCNVAHPASKTKVDKPVPKRENGRVPRPPDCPKCPAPEMLGGPSVFIFPPKPKDTLLIARTPEVTCVVVDLDPEDPEVQISWFVDGKQMQTAKTQPREEQFNGTYRVVSVLPIGHQDWLKGKQFTCKVNNKALPSPIERTISKARGQAHQPSVYVLPPSREELSKNTVSLTCLIKDFFPPDIDVEWQSNGQQEPESKYRTTPPQLDEDGSYFLYSKLSVDKSRWQRGDTFICAVMHEALHNHYTQKSLSHSPGGGGGSGGGGSGGGGSGGGGSGGGGSPKRENGRVPRPPDCPKCPAPEMLGGPSVFIFPPKPKDTLLIARTPEVTCVVVDLDPEDPEVQISWFVDGKQMQTAKTQPREEQFNGTYRVVSVLPIGHQDWLKGKQFTCKVNNKALPSPIERTISKARGQAHQPSVYVLPPSREELSKNTVSLTCLIKDFFPPDIDVEWQSNGQQEPESKYRTTPPQLDEDGSYFLYSKLSVDKSRWQRGDTFICAVMHEALHNHYTQKSLSHSPGGGGGSGPPGISKEGPPGDPGLPGKDGDHGKPGIQGQPGPPGICDPSLCFSVIVGRDPFRKGPNY

SEQ ID NO: 9 - protein, 5 aa, Artificial Sequence
  Synthesized
GGGGS

SEQ ID NO: 10 - protein, 25 aa, Artificial Sequence
  Synthesized in La
GGGGSGGGGSGGGGSGGGGSGGGGS